European Patent Specification EP 3 299 461 B1, published March 29, 2023. Title: NOVEL ANTI-HUMAN NGF ANTIBODY FAB FRAGMENT. Applicant: Astellas Pharma Inc. The sequence listing filed with the application follows.

SEQUENCE LISTING (12 sequences)

SEQ ID NO: 1 - DNA, 675 bp, Artificial Sequence
  DNA encoding h1f.6 heavy chain fragment
caggtgcagctacagcagtggggcgcaggactgttgaagccttcggagaccctgtccctcacctgcgctgtctatggtgggtccttcagtggttactactggagctgggtccgccagcccccagggaaggggctggagtggattggggaaatcgaccatagtggaagcaccaacaacaacccgtccctcaagagtcgagtcaccatatcagtaggcacgtccaagaaccagttctccctgaagctgagctctgtgaccgccgcggacacggctgtgtattactgttcgagagatgggggccccgaatcggggatgggggcttttgatatctggggccaagggacaatggtcaccgtctcctcagcctccaccaagggcccatcggtcttccccctggcaccctcctccaagagcacctctgggggcacagcggccctgggctgcctggtcaaggactacttccccgaaccggtgacggtgtcgtggaactcaggcgccctgaccagcggcgtgcacaccttcccggctgtcctacagtcctcaggactctactcccttagtagcgtggtgaccgtgccctccagcagcttgggcacccagacctacatctgcaacgtgaatcacaagcccagcaacaccaaggtggacaagaaagttgagcccaaatcttgtgac

SEQ ID NO: 2 - DNA, 672 bp, Artificial Sequence
  DNA encoding h1f.7 heavy chain fragment
caggtgcagctacagcagtggggcgcaggactgttgaagccttcggagaccctgtccctcacctgcgctgtctatggtgggtccttcagtggttactactggagctgggtccgccagcccccagggaaggggctggagtggattggggaaatcgaccatagtggaagcaccaacaacaacccgtccctcaagagtcgagtcaccatatcagtaggcacgtccaagaaccagttctccctgaagctgagctctgtgaccgccgcggacacggctgtgtattactgttcgagagatgggggccccgaatcggggatgggggcttttgatatctggggccaagggacaatggtcaccgtctcctcagcctccaccaagggcccatcggtcttccccctggcaccctcctccaagagcacctctgggggcacagcggccctgggctgcctggtcaaggactacttccccgaaccggtgacggtgtcgtggaactcaggcgccctgaccagcggcgtgcacaccttcccggctgtcctacagtcctcaggactctactcccttagtagcgtggtgaccgtgccctccagcagcttgggcacccagacctacatctgcaacgtgaatcacaagcccagcaacaccaaggtggacaagaaagttgagcccaaatcttgt

SEQ ID NO: 3 - DNA, 678 bp, Artificial Sequence
  DNA encoding h1f.8 heavy chain fragment
caggtgcagctacagcagtggggcgcaggactgttgaagccttcggagaccctgtccctcacctgcgctgtctatggtgggtccttcagtggttactactggagctgggtccgccagcccccagggaaggggctggagtggattggggaaatcgaccatagtggaagcaccaacaacaacccgtccctcaagagtcgagtcaccatatcagtaggcacgtccaagaaccagttctccctgaagctgagctctgtgaccgccgcggacacggctgtgtattactgttcgagagatgggggccccgaatcggggatgggggcttttgatatctggggccaagggacaatggtcaccgtctcctcagcctccaccaagggcccatcggtcttccccctggcaccctcctccaagagcacctctgggggcacagcggccctgggctgcctggtcaaggactacttccccgaaccggtgacggtgtcgtggaactcaggcgccctgaccagcggcgtgcacaccttcccggctgtcctacagtcctcaggactctactcccttagtagcgtggtgaccgtgccctccagcagcttgggcacccagacctacatctgcaacgtgaatcacaagcccagcaacaccaaggtggacaagaaagttgagcccaaatcttgtgcagcc

SEQ ID NO: 4 - DNA, 657 bp, Artificial Sequence
  DNA encoding 1-15(N52D-A)-Fab' fragment light chain
gatattgtgatgactcagtctccactctccctgcccgtcacccctggagagccggcctccatctcctgcaggtctagtcagagcctcctgcatagtaatggattcaactatttgggttggtacctgcagaagccagggcagtctccacagctcctgatctatttgggttctaatcgggcctccggggtccctgacaggttcagtggcagtggatcaggcacagattttactctgaaaatcagcagagtggaggctgaggatgttggggtttattactgcatgcaagctctacaaactccgtacacttttggccaggggaccaagctggagatcaaacggactgtggctgcaccatctgtcttcatcttcccgccatctgatgagcagttgaaatctggaactgcctctgttgtgtgcctgctgaataacttctatcccagagaggccaaagtacagtggaaggtggataacgccctccaatcgggtaactcccaggagagtgtcacagagcaggacagcaaggacagcacctacagcctcagcagcaccctgacgctgagcaaagcagactacgagaaacacaaagtctacgcctgcgaagtcacccatcagggcctgagctcgcccgtcacaaagagcttcaacaggggagagtgt

SEQ ID NO: 5 - protein, 225 aa, Artificial Sequence
  h1f.6 heavy chain fragment
QVQLQQWGAGLLKPSETLSLTCAVYGGSFSGYYWSWVRQPPGKGLEWIGEIDHSGSTNNNPSLKSRVTISVGTSKNQFSLKLSSVTAADTAVYYCSRDGGPESGMGAFDIWGQGTMVTVSSASTKGPSVFPLAPSSKSTSGGTAALGCLVKDYFPEPVTVSWNSGALTSGVHTFPAVLQSSGLYSLSSVVTVPSSSLGTQTYICNVNHKPSNTKVDKKVEPKSCD

SEQ ID NO: 6 - protein, 224 aa, Artificial Sequence
  h1f.7 heavy chain fragment
QVQLQQWGAGLLKPSETLSLTCAVYGGSFSGYYWSWVRQPPGKGLEWIGEIDHSGSTNNNPSLKSRVTISVGTSKNQFSLKLSSVTAADTAVYYCSRDGGPESGMGAFDIWGQGTMVTVSSASTKGPSVFPLAPSSKSTSGGTAALGCLVKDYFPEPVTVSWNSGALTSGVHTFPAVLQSSGLYSLSSVVTVPSSSLGTQTYICNVNHKPSNTKVDKKVEPKSC

SEQ ID NO: 7 - protein, 226 aa, Artificial Sequence
  h1f.8 heavy chain fragment
QVQLQQWGAGLLKPSETLSLTCAVYGGSFSGYYWSWVRQPPGKGLEWIGEIDHSGSTNNNPSLKSRVTISVGTSKNQFSLKLSSVTAADTAVYYCSRDGGPESGMGAFDIWGQGTMVTVSSASTKGPSVFPLAPSSKSTSGGTAALGCLVKDYFPEPVTVSWNSGALTSGVHTFPAVLQSSGLYSLSSVVTVPSSSLGTQTYICNVNHKPSNTKVDKKVEPKSCAA

SEQ ID NO: 8 - protein, 219 aa, Artificial Sequence
  1-15(N52D-A)-Fab' fragment light chain
DIVMTQSPLSLPVTPGEPASISCRSSQSLLHSNGFNYLGWYLQKPGQSPQLLIYLGSNRASGVPDRFSGSGSGTDFTLKISRVEAEDVGVYYCMQALQTPYTFGQGTKLEIKRTVAAPSVFIFPPSDEQLKSGTASVVCLLNNFYPREAKVQWKVDNALQSGNSQESVTEQDSKDSTYSLSSTLTLSKADYEKHKVYACEVTHQGLSSPVTKSFNRGEC

SEQ ID NO: 9 - DNA, 363 bp, Artificial Sequence
  VH gene of anti-human NGF antibody
  CDS (1)..(363)
caggtgcagctacagcagtggggcgcaggactgttgaagccttcggagaccctgtccctcacctgcgctgtctatggtgggtccttcagtggttactactggagctgggtccgccagcccccagggaaggggctggagtggattggggaaatcgaccatagtggaagcaccaacaacaacccgtccctcaagagtcgagtcaccatatcagtaggcacgtccaagaaccagttctccctgaagctgagctctgtgaccgccgcggacacggctgtgtattactgttcgagagatgggggccccgaatcggggatgggggcttttgatatctggggccaagggacaatggtcaccgtctcctca

SEQ ID NO: 10 - protein, 121 aa, Artificial Sequence
  Synthetic Construct
QVQLQQWGAGLLKPSETLSLTCAVYGGSFSGYYWSWVRQPPGKGLEWIGEIDHSGSTNNNPSLKSRVTISVGTSKNQFSLKLSSVTAADTAVYYCSRDGGPESGMGAFDIWGQGTMVTVSS

SEQ ID NO: 11 - DNA, 339 bp, Artificial Sequence
  VL gene of anti-human NGF antibody
  CDS (1)..(339)
gatattgtgatgactcagtctccactctccctgcccgtcacccctggagagccggcctccatctcctgcaggtctagtcagagcctcctgcatagtaatggattcaactatttgggttggtacctgcagaagccagggcagtctccacagctcctgatctatttgggttctaatcgggcctccggggtccctgacaggttcagtggcagtggatcaggcacagattttactctgaaaatcagcagagtggaggctgaggatgttggggtttattactgcatgcaagctctacaaactccgtacacttttggccaggggaccaagctggagatcaaacgg

SEQ ID NO: 12 - protein, 113 aa, Artificial Sequence
  Synthetic Construct
DIVMTQSPLSLPVTPGEPASISCRSSQSLLHSNGFNYLGWYLQKPGQSPQLLIYLGSNRASGVPDRFSGSGSGTDFTLKISRVEAEDVGVYYCMQALQTPYTFGQGTKLEIKR